European Patent Specification EP 3 484 496 B1, published December 27, 2023. Title: METHODS AND COMPOSITION FOR PRODUCING AND USING IMMUNE CELLS AND STEM CELLS FOR CELL-BASED THERAPIES. Applicant: University of Southern California. Application Not yet assigned. The sequence listing filed with the application follows.

SEQUENCE LISTING (1 sequence)

SEQ ID NO: 1 - DNA, 9659 bp, Artificial Sequence
  Vector - pLenti-EF1a-FMC63(vL-vH)-Myc-BBz-T2A-Pac-A13
aatgtagtcttatgcaatactcttgtagtcttgcaacatggtaacgatgagttagcaacatgccttacaaggagagaaaaagcaccgtgcatgccgattggtggaagtaaggtggtacgatcgtgccttattaggaaggcaacagacgggtctgacatggattggacgaaccactgaattgccgcattgcagagatattgtatttaagtgcctagctcgatacataaacgggtctctctggttagaccagatctgagcctgggagctctctggctaactagggaacccactgcttaagcctcaataaagcttgccttgagtgcttcaagtagtgtgtgcccgtctgttgtgtgactctggtaactagagatccctcagacccttttagtcagtgtggaaaatctctagcagtggcgcccgaacagggacttgaaagcgaaagggaaaccagaggagctctctcgacgcaggactcggcttgctgaagcgcgcacggcaagaggcgaggggcggcgactggtgagtacgccaaaaattttgactagcggaggctagaaggagagagatgggtgcgagagcgtcagtattaagcgggggagaattagatcgcgatgggaaaaaattcggttaaggccagggggaaagaaaaaatataaattaaaacatatagtatgggcaagcagggagctagaacgattcgcagttaatcctggcctgttagaaacatcagaaggctgtagacaaatactgggacagctacaaccatcccttcagacaggatcagaagaacttagatcattatataatacagtagcaaccctctattgtgtgcatcaaaggatagagataaaagacaccaaggaagctttagacaagatagaggaagagcaaaacaaaagtaagaccaccgcacagcaagcggccgctgatcttcagacctggaggaggagatatgagggacaattggagaagtgaattatataaatataaagtagtaaaaattgaaccattaggagtagcacccaccaaggcaaagagaagagtggtgcagagagaaaaaagagcagtgggaataggagctttgttccttgggttcttgggagcagcaggaagcactatgggcgcagcgtcaatgacgctgacggtacaggccagacaattattgtctggtatagtgcagcagcagaacaatttgctgagggctattgaggcgcaacagcatctgttgcaactcacagtctggggcatcaagcagctccaggcaagaatcctggctgtggaaagatacctaaaggatcaacagctcctggggatttggggttgctctggaaaactcatttgcaccactgctgtgccttggaatgctagttggagtaataaatctctggaacagatttggaatcacacgacctggatggagtgggacagagaaattaacaattacacaagcttaatacactccttaattgaagaatcgcaaaaccagcaagaaaagaatgaacaagaattattggaattagataaatgggcaagtttgtggaattggtttaacataacaaattggctgtggtatataaaattattcataatgatagtaggaggcttggtaggtttaagaatagtttttgctgtactttctatagtgaatagagttaggcagggatattcaccattatcgtttcagacccacctcccaaccccgaggggacccgacaggcccgaaggaatagaagaagaaggtggagagagagacagagacagatccattcgattagtgaacggatctcgacggtatcggttaacttttaaaagaaaaggggggattggggggtacagtgcaggggaaagaatagtagacataatagcaacagacatacaaactaaagaattacaaaaacaaattacaaaattcaaaattttatcgataagctttgcaaagatggataaagttttaaacagagaggaatctttgcagctaatggaccttctaggtcttgaaaggagtgcctcgtgaggctccggtgcccgtcagtgggcagagcgcacatcgcccacagtccccgagaagttggggggaggggtcggcaattgaaccggtgcctagagaaggtggcgcggggtaaactgggaaagtgatgtcgtgtactggctccgcctttttcccgagggtgggggagaaccgtatataagtgcagtagtcgccgtgaacgttctttttcgcaacgggtttgccgccagaacacaggtaagtgccgtgtgtggttcccgcgggcctggcctctttacgggttatggcccttgcgtgccttgaattacttccacctggctgcagtacgtgattcttgatcccgagcttcgggttggaagtgggtgggagagttcgaggccttgcgcttaaggagccccttcgcctcgtgcttgagttgaggcctggcctgggcgctggggccgccgcgtgcgaatctggtggcaccttcgcgcctgtctcgctgctttcgataagtctctagccatttaaaatttttgatgacctgctgcgacgctttttttctggcaagatagtcttgtaaatgcgggccaagatctgcacactggtatttcggtttttggggccgcgggcggcgacggggcccgtgcgtcccagcgcacatgttcggcgaggcggggcctgcgagcgcggccaccgagaatcggacgggggtagtctcaagctggccggcctgctctggtgcctggcctcgcgccgccgtgtatcgccccgccctgggcggcaaggctggcccggtcggcaccagttgcgtgagcggaaagatggccgcttcccggccctgctgcagggagctcaaaatggaggacgcggcgctcgggagagcgggcgggtgagtcacccacacaaaggaaaagggcctttccgtcctcagccgtcgcttcatgtgactccacggagtaccgggcgccgtccaggcacctcgattagttctcgaccttttggagtacgtcgtctttaggttggggggaggggttttatgcgatggagtttccccacactgagtgggtggagactgaagttaggccagcttggcacttgatgtaattctccttggaatttgccctttttgagtttggatcttggttcattctcaagcctcagacagtggttcaaagtttttttcttccatttcaggtgtcgtgaggaattagcttggtactaatacgactcactatagggagacccaagctggctagttaagcttgatatcgaattcctgcagcccgggggatctgctagcatggccttaccagtgaccgccttgctcctgccgctggccttgctgctccacgccgccaggccggacatccagatgacacagactacatcctccctgtctgcctctctgggagacagagtcaccatcagttgcagggcaagtcaggacattagtaaatatttaaattggtatcagcagaaaccagatggaactgttaaactcctgatctaccatacatcaagattacactcaggagtcccatcaaggttcagtggcagtgggtctggaacagattattctctcaccattagcaacctggagcaagaagatattgccacttacttttgccaacagggtaatacgcttccgtacacgttcggaggggggaccaagctggagatcacaggtggcggtggctcgggcggtggtgggtcgggtggcggcggatctgaggtgaaactgcaggagtcaggacctggcctggtggcgccctcacagagcctgtccgtcacatgcactgtctcaggggtctcattacccgactatggtgtaagctggattcgccagcctccacgaaagggtctggagtggctgggagtaatatggggtagtgaaaccacatactataattcagctctcaaatccagactgaccatcatcaaggacaactccaagagccaagttttcttaaaaatgaacagtctgcaaactgatgacacagccatttactactgtgccaaacattattactacggtggtagctatgctatggactactggggtcaaggaacctcagtcaccgtctcctcacgcgtagagcagaaactgatctcggaagaggatctggcgaagcccaccacgacgccagcgccgcgaccaccaacaccggcgcccaccatcgcgtcgcagcccctgtccctgcgcccagaggcgtgccggccagcggcggggggcgcagtgcacacgagggggctggacttcgcctgtgacatctacatctgggcgcccttggccgggacttgtggggtccttctcctgtcactggttatcaccctttactgcaaacggggcagaaagaaactcctgtatatattcaaacaaccatttatgagaccagtacaaactactcaagaggaagatggctgtagctgccgatttccagaagaagaagaaggaggatgtgaactgagagtgaagttcagcaggagcgcagacgcccccgcgtaccagcagggccagaaccagctctataacgagctgaatctaggacgaagagaggagtacgatgttttggacaagagacgtggccgggaccctgagatggggggaaagccgagaaggaagaaccctcaggaaggcctgtacaatgaactgcagaaagataagatggcggaggcctacagtgagattgggatgaaaggcgagcgccggaggggcaaggggcacgatggcctttaccagggtctcagtacagccaccaaggacacctacgacgcccttcacatgcaggccctgccccctcgctctagtggctccggcgagggcagaggaagtctactaacctgcggagatgtggaagaaaatcctggcccacatatgaccgagtacaagcccacggtgcgcctcgccacccgcgacgacgtccccagggccgtacgcaccctcgccgccgcgttcgccgactaccccgccacgcgccacaccgtcgatccggaccgccacatcgagcgggtcaccgagctgcaagaactcttcctcacgcgcgtcgggctcgacatcggcaaggtgtgggtcgcggacgacggcgccgcggtggcggtctggaccacgccggagagcgtcgaagcgggggcggtgttcgccgagatcggcccgcgcatggccgagttgagcggttcccggctggccgcgcagcaacagatggaaggcctcctggcgccgcaccggcccaaggagcccgcgtggttcctggccaccgtcggcgtctcgcccgaccaccagggcaagggtctgggcagcgccgtcgtgctccccggagtggaggcggccgagcgcgccggggtgcccgccttcctggagacctccgcgccccgcaacctccccttctacgagcggctcggcttcaccgtcaccgccgacgtcgaggtgcccgaaggaccgcgcacctggtgcatgacccgcaagcccggtgcctgagtcgactccggatgatcagggccctgtacagatatcgacaatcaacctctggattacaaaatttgtgaaagattgactggtattcttaactatgttgctccttttacgctatgtggatacgctgctttaatgcctttgtatcatgctattgcttcccgtatggctttcattttctcctccttgtataaatcctggttgctgtctctttatgaggagttgtggcccgttgtcaggcaacgtggcgtggtgtgcactgtgtttgctgacgcaacccccactggttggggcattgccaccacctgtcagctcctttccgggactttcgctttccccctccctattgccacggcggaactcatcgccgcctgccttgcccgctgctggacaggggctcggctgttgggcactgacaattccgtggtgttgtcggggaagctgacgtcctttccatggctgctcgcctgtgttgccacctggattctgcgcgggacgtccttctgctacgtcccttcggccctcaatccagcggaccttccttcccgcggcctgctgccggctctgcggcctcttccgcgtcttcgccttcgccctcagacgagtcggatctccctttgggccgcctccccgcctggaattcgagctcggtacctttaagaccaatgacttacaaggcagctgtagatcttagccactttttaaaagaaaaggggggactggaagggctaattcactcccaacgaagacaagatctgctttttgcttgtactgggtctctctggttagaccagatctgagcctgggagctctctggctaactagggaacccactgcttaagcctcaataaagcttgccttgagtgcttcaagtagtgtgtgcccgtctgttgtgtgactctggtaactagagatccctcagacccttttagtcagtgtggaaaatctctagcagtagtagttcatgtcatcttattattcagtatttataacttgcaaagaaatgaatatcagagagtgagaggaacttgtttattgcagcttataatggttacaaataaagcaatagcatcacaaatttcacaaataaagcatttttttcactgcattctagttgtggtttgtccaaactcatcaatgtatcttatcatgtctggctctagctatcccgcccctaactccgcccatcccgcccctaactccgcccagttccgcccattctccgccccatggctgactaattttttttatttatgcagaggccgaggccgcctcggcctctgagctattccagaagtagtgaggaggcttttttggaggcctagggacgtacccaattcgccctatagtgagtcgtattacgcgcgctcactggccgtcgttttacaacgtcgtgactgggaaaaccctggcgttacccaacttaatcgccttgcagcacatccccctttcgccagctggcgtaatagcgaagaggcccgcaccgatcgcccttcccaacagttgcgcagcctgaatggcgaatgggacgcgccctgtagcggcgcattaagcgcggcgggtgtggtggttacgcgcagcgtgaccgctacacttgccagcgccctagcgcccgctcctttcgctttcttcccttcctttctcgccacgttcgccggctttccccgtcaagctctaaatcgggggctccctttagggttccgatttagtgctttacggcacctcgaccccaaaaaacttgattagggtgatggttcacgtagtgggccatcgccctgatagacggtttttcgccctttgacgttggagtccacgttctttaatagtggactcttgttccaaactggaacaacactcaaccctatctcggtctattcttttgatttataagggattttgccgatttcggcctattggttaaaaaatgagctgatttaacaaaaatttaacgcgaattttaacaaaatattaacgcttacaatttaggtggcacttttcggggaaatgtgcgcggaacccctatttgtttatttttctaaatacattcaaatatgtatccgctcatgagacaataaccctgataaatgcttcaataatattgaaaaaggaagagtatgagtattcaacatttccgtgtcgcccttattcccttttttgcggcattttgccttcctgtttttgctcacccagaaacgctggtgaaagtaaaagatgctgaagatcagttgggtgcacgagtgggttacatcgaactggatctcaacagcggtaagatccttgagagttttcgccccgaagaacgttttccaatgatgagcacttttaaagttctgctatgtggcgcggtattatcccgtattgacgccgggcaagagcaactcggtcgccgcatacactattctcagaatgacttggttgagtactcaccagtcacagaaaagcatcttacggatggcatgacagtaagagaattatgcagtgctgccataaccatgagtgataacactgcggccaacttacttctgacaacgatcggaggaccgaaggagctaaccgcttttttgcacaacatgggggatcatgtaactcgccttgatcgttgggaaccggagctgaatgaagccataccaaacgacgagcgtgacaccacgatgcctgtagcaatggcaacaacgttgcgcaaactattaactggcgaactacttactctagcttcccggcaacaattaatagactggatggaggcggataaagttgcaggaccacttctgcgctcggcccttccggctggctggtttattgctgataaatctggagccggtgagcgtgggtctcgcggtatcattgcagcactggggccagatggtaagccctcccgtatcgtagttatctacacgacggggagtcaggcaactatggatgaacgaaatagacagatcgctgagataggtgcctcactgattaagcattggtaactgtcagaccaagtttactcatatatactttagattgatttaaaacttcatttttaatttaaaaggatctaggtgaagatcctttttgataatctcatgaccaaaatcccttaacgtgagttttcgttccactgagcgtcagaccccgtagaaaagatcaaaggatcttcttgagatcctttttttctgcgcgtaatctgctgcttgcaaacaaaaaaaccaccgctaccagcggtggtttgtttgccggatcaagagctaccaactctttttccgaaggtaactggcttcagcagagcgcagataccaaatactgttcttctagtgtagccgtagttaggccaccacttcaagaactctgtagcaccgcctacatacctcgctctgctaatcctgttaccagtggctgctgccagtggcgataagtcgtgtcttaccgggttggactcaagacgatagttaccggataaggcgcagcggtcgggctgaacggggggttcgtgcacacagcccagcttggagcgaacgacctacaccgaactgagatacctacagcgtgagctatgagaaagcgccacgcttcccgaagggagaaaggcggacaggtatccggtaagcggcagggtcggaacaggagagcgcacgagggagcttccagggggaaacgcctggtatctttatagtcctgtcgggtttcgccacctctgacttgagcgtcgatttttgtgatgctcgtcaggggggcggagcctatggaaaaacgccagcaacgcggcctttttacggttcctggccttttgctggccttttgctcacatgttctttcctgcgttatcccctgattctgtggataaccgtattaccgcctttgagtgagctgataccgctcgccgcagccgaacgaccgagcgcagcgagtcagtgagcgaggaagcggaagagcgcccaatacgcaaaccgcctctccccgcgcgttggccgattcattaatgcagctggcacgacaggtttcccgactggaaagcgggcagtgagcgcaacgcaattaatgtgagttagctcactcattaggcaccccaggctttacactttatgcttccggctcgtatgttgtgtggaattgtgagcggataacaatttcacacaggaaacagctatgaccatgattacgccaagcgcgcaattaaccctcactaaagggaacaaaagctggagctgcaagctt